European Patent Specification EP 3 266 872 B1, published May 17, 2023. Title: Novel anti-PAD4 antibody. Applicant: Public University Corporation Yokohama City University Public University Corporation Nagoya City University Pharma Foods International Co., Ltd. The sequence listing filed with the application follows.

SEQUENCE LISTING (197 sequences)

SEQ ID NO: 1 - protein, 17 aa, Artificial Sequence
  peptide antigen
EENMDDQWMQDEMEIGY

SEQ ID NO: 2 - protein, 663 aa, Homo sapiens
MAQGTLIRVTPEQPTHAVCVLGTLTQLDICSSAPEDCTSFSINASPGVVVDIAHGPPAKKKSTGSSTWPLDPGVEVTLTMKVASGSTGDQKVQISYYGPKTPPVKALLYLTGVEISLCADITRTGKVKPTRAVKDQRTWTWGPCGQGAILLVNCDRDNLESSAMDCEDDEVLDSEDLQDMSLMTLSTKTPKDFFTNHTLVLHVARSEMDKVRVFQATRGKLSSKCSVVLGPKWPSHYLMVPGGKHNMDFYVEALAFPDTDFPGLITLTISLLDTSNLELPEAVVFQDSVVFRVAPWIMTPNTQPPQEVYACSIFENEDFLKSVTTLAMKAKCKLTICPEEENMDDQWMQDEMEIGYIQAPHKTLPVVFDSPRNRGLKEFPIKRVMGPDFGYVTRGPQTGGISGLDSFGNLEVSPPVTVRGKEYPLGRILFGDSCYPSNDSRQMHQALQDFLSAQQVQAPVKLYSDWLSVGHVDEFLSFVPAPDRKGFRLLLASPRSCYKLFQEQQNEGHGEALLFEGIKKKKQQKIKNILSNKTLREHNSFVERCIDWNRELLKRELGLAESDIIDIPQLFKLKEFSKAEAFFPNMVNMLVLGKHLGIPKPFGPVINGRCCLEEKVCSLLEPLGLQCTFINDFFTYHIRHGEVHCGTNVRRKPFSFKWWNMVP

SEQ ID NO: 3 - protein, 119 aa, chicken
AVTLDESGGGLQTPGGALSLVCKASGFDFSSYGMGWMRQAPGKGLEYVAAIRNDGSWTGYGAAVKGHATISRDNGQSTVRLQLNNLRAEDTGTYYCAKTTGSRGGSIDAWGHGTEVIVS

SEQ ID NO: 4 - protein, 119 aa, chicken
AVTLDESGGGLQTPGGTLSLVCKGSGFTFSSYGMGWMRQAPGKGLEYVAAIRNDGSWTGYGSAVKGRATISRDNGQSTVRLQLNNLRAEDTATYYCAKTSGSSGGSVDAWGHGTEVIVS

SEQ ID NO: 5 - protein, 119 aa, chicken
AVTLDESGGGLQTPGGALSLVCKASGFTFSSYGMEWVRQAPGKGLEYVAAIRNDGSWTGYGAAVKGRATISRDDGQSTLRLQLNNLRAEDTATYYCAKTTGSSGGSIDAWGHGTEVIVS

SEQ ID NO: 6 - protein, 119 aa, chicken
AVTLDESGGGLQTPGGALSLVCKASGFTFSTYAMGWMRQAPGKGLEYVAAIRNDGSWTGYGAAVKGRATILRDNGQSTVRLQLSNLRAEDTGTYYCAKYTGSSGGSIGAWGHGTEVIVS

SEQ ID NO: 7 - protein, 119 aa, chicken; identical to SEQ ID NO: 6

SEQ ID NO: 8 - protein, 119 aa, chicken; identical to SEQ ID NO: 6

SEQ ID NO: 9 - DNA, 357 bp, chicken
gcggtgacgttggacgagtccgggggcggcctccagacgcccggaggagcgctcagcctcgtctgcaaggcctccgggtttgacttcagtagttatggcatgggatggatgcgccaggcgcccggcaaggggctggaatacgttgcagctattaggaatgatggcagttggacaggctacggggcggcggtgaagggccatgccaccatctcgagggacaacgggcagagcacagtgaggctgcagctgaacaacctcagggctgaggacaccggcacctactactgcgccaaaactactggtagtcgtggtggtagcatcgacgcatggggccacgggaccgaagtcatcgtctcc

SEQ ID NO: 10 - DNA, 357 bp, chicken
gcggtgacgttggacgagtccgggggcggcctccagacgcccggaggaacgctcagcctcgtctgcaagggctccgggttcaccttcagtagttatggcatgggatggatgcgccaggcgcccggcaaggggctggaatacgttgcagctatcaggaatgatggtagttggacaggctacgggtcggcggtgaagggccgtgccaccatctcgagggacaacgggcagagcacagtgaggctgcagttgaacaacctcagggctgaggacaccgccacctactactgcgccaaaactagtggtagtagtggtggtagcgtcgacgcatggggccacgggaccgaagtcatcgtctcc

SEQ ID NO: 11 - protein, 357 aa, chicken
GCGGTGACGTTGGACGAGTCCGGGGGCGGCCTCCAGACGCCCGGAGGAGCGCTCAGCCTCGTCTGCAAGGCCTCCGGGTTCACCTTCAGTAGTTATGGCATGGAGTGGGTGCGACAGGCGCCCGGCAAGGGGCTGGAATACGTTGCAGCTATTAGGAATGATGGTAGTTGGACAGGCTACGGGGCGGCGGTGAAGGGCCGTGCCACCATCTCGAGGGACGACGGGCAGAGCACACTGAGGCTGCAGCTGAACAACCTCAGGGCTGAGGACACCGCCACCTACTACTGCGCCAAAACTACTGGTAGTAGTGGTGGTAGCATCGACGCATGGGGCCACGGGACCGAAGTCATCGTCTCC

SEQ ID NO: 12 - DNA, 357 bp, chicken
gcggtgacgttggacgagtccgggggcggcctccagacgcccggaggagcgctcagcctcgtctgcaaggcctccgggttcaccttcagtacttatgccatgggttggatgcgccaggcacccggcaaggggctggagtatgtcgcagctattaggaatgatggtagttggacaggctacggggcggcggtgaagggccgtgccaccatcttgagggacaacgggcagagcacagtgaggctgcagctgagcaacctcagggctgaggacaccggcacctactactgcgccaaatatactggtagtagtggtggtagcatcggcgcatggggccacgggaccgaagtcatcgtctcc

SEQ ID NO: 13 - DNA, 357 bp, chicken
gccgtgacgttggacgagtccgggggcggcctccagacgcccggaggagcgctcagcctcgtctgcaaggcctccgggttcaccttcagtacttatgccatgggttggatgcgccaggcacccggcaaggggctggagtatgtcgcagctattaggaatgatggtagttggacaggctacggggcggcggtgaagggccgtgccaccatcttgagggacaacgggcagagcacagtgaggctgcagctgagcaacctcagggctgaggacaccggcacctactactgcgccaaatatactggtagtagtggtggtagcatcggcgcatggggccacgggaccgaagtcatcgtctcc

SEQ ID NO: 14 - DNA, 357 bp, chicken; identical to SEQ ID NO: 12

SEQ ID NO: 15 - protein, 103 aa, chicken
ASTQPSSVSANLGGTVEITCSGGGRYYYGWYQQKSPGSAPVTVIYANDKRPSDIPSRFSGSKSGSTGTLTITGVQAEDEAVYFCGSAETSSYVFGAGTTLTVL

SEQ ID NO: 16 - protein, 103 aa, chicken; identical to SEQ ID NO: 15

SEQ ID NO: 17 - protein, 103 aa, chicken
ASTQPSSVSANLGETVKITCSGGGNYYYGWYQQKSPGSAPVTLIYANDKRPSNIPSRFSGSKSGSTGTLTITGVQAEDEAVYFCGTADTGKYVFGAGTTLTVL

SEQ ID NO: 18 - protein, 104 aa, chicken
ASTQPSSVSANLGGTVEITCSGGNRNYYYGWYQQKSPGSAPVTLIYANDKRPSNIPSRFSGSKSGSTGTLTITGVQAEDEAVYFCGTADTGKYVFGAGTTLTVL

SEQ ID NO: 19 - protein, 103 aa, chicken
AVTQPASVSANLGGTVEITCSGGGRYYYGWYQQKSPGSAPVTVIYANDKRPSDIPSRFSGSKSGSTGTLTITGVQAEDEAVYFCGSAETSSYVFGAGTTLTVL

SEQ ID NO: 20 - protein, 104 aa, chicken
ASTQPSSVSANPGGTVEITCSGGSGRYYYGWYQQKSPGSAPVTVIYSSTHRPSNIPSRFSGSKSGSTATLTITGVQAEDEAVYFCGTADSSSYVFGAGTTLTVL

SEQ ID NO: 21 - DNA, 309 bp, chicken
gctagcactcagccgtcctcggtgtcagcaaacctgggaggaaccgtcgagatcacctgctccgggggtggcaggtactattatggctggtaccagcagaagtctcctggcagtgcccctgtcactgtgatctatgctaacgacaagagaccctcggacatcccttcacgattctccggttccaaatccggctccacgggcacattgaccatcactggggtccaagccgaggacgaggctgtctatttctgtgggagtgcagagaccagcagctatgtatttggggccgggacaaccctgaccgtccta

SEQ ID NO: 22 - DNA, 309 bp, chicken
gctagcactcagccgtcctcggtgtcagcaaacctgggaggaaccgtcgagatcacctgctccgggggtggcaggtactattatggctggtaccagcagaagtctcctggcagtgcccctgtcactgtgatctatgctaacgacaagagaccctcggacatcccttcacgattctccggttccaaatccggctccacgggcacattgaccatcactggggtccaagccgaagacgaggctgtctatttctgtgggagtgcagagaccagcagctatgtatttggggccgggacaaccctgaccgtccta

SEQ ID NO: 23 - DNA, 309 bp, chicken
gctagcactcagccgtcctcggtgtcagcaaacctgggagaaaccgtcaagatcacctgctccgggggtggcaattattactatggctggtaccagcagaagtcacctggcagtgcccctgtcactctgatctatgctaacgacaagagaccctcgaacatcccttcacgattctccggttccaaatccggctccacaggcacattaaccatcactggggtccaagccgaggacgaggctgtctatttctgtgggaccgcagacaccgggaagtatgtatttggggccgggacaaccctgaccgtccta

SEQ ID NO: 24 - DNA, 312 bp, chicken
gctagcactcagccgtcctcggtgtcagcaaacctgggaggaaccgtcgagatcacctgctccggggggaataggaactactactatggctggtaccagcagaagtcacctggcagtgcccctgtcactctgatctatgctaacgacaagagaccctcgaacatcccttcacgattctccggttccaaatccggctccacaggcacattaaccatcactggggtccaagccgaggacgaggctgtctatttctgtgggaccgcagacaccgggaagtatgtatttggggccgggacaaccctgaccgtccta

SEQ ID NO: 25 - DNA, 309 bp, chicken
gcagtgactcagccggcctcagtgtcagcaaacctgggaggaaccgtcgagatcacctgctccgggggtggcaggtactattatggctggtaccagcagaagtctcctggcagtgcccctgtcactgtgatctatgctaacgacaagagaccctcggacatcccttcacgattctccggttccaaatccggctccacgggcacattgaccatcactggggtccaagcagaggacgaggctgtctatttctgtgggagtgcagagaccagcagctatgtatttggggccgggacaaccctgaccgtcctc

SEQ ID NO: 26 - DNA, 312 bp, chicken
gctagcactcagccgtcctcggtgtcagcaaacccaggaggaaccgtcgagatcacctgctccgggggtagtggcaggtactattatggctggtaccagcagaagtctcctggcagtgcccctgtcactgtgatctatagcagcacccacagaccctcaaacatcccttcacgattctccggttccaaatccggctccacggccacattaaccatcactggggtccaagccgaggacgaggctgtctatttctgtgggactgcagacagcagcagctatgtctttggggccgggacaaccctgaccgtccta

SEQ ID NO: 27 - protein, 17 aa, Artificial Sequence
  peptide
AENMDDQWMQDEMEIGY

SEQ ID NO: 28 - protein, 17 aa, Artificial Sequence
  peptide
EANMDDQWMQDEMEIGY

SEQ ID NO: 29 - protein, 17 aa, Artificial Sequence
  peptide
EEAMDDQWMQDEMEIGY

SEQ ID NO: 30 - protein, 17 aa, Artificial Sequence
  peptide
EENADDQWMQDEMEIGY

SEQ ID NO: 31 - protein, 17 aa, Artificial Sequence
  peptide
EENMADQWMQDEMEIGY

SEQ ID NO: 32 - protein, 17 aa, Artificial Sequence
  peptide
EENMDAQWMQDEMEIGY

SEQ ID NO: 33 - protein, 17 aa, Artificial Sequence
  peptide
EENMDDAWMQDEMEIGY

SEQ ID NO: 34 - protein, 17 aa, Artificial Sequence
  peptide
EENMDDQAMQDEMEIGY

SEQ ID NO: 35 - protein, 17 aa, Artificial Sequence
  peptide
EENMDDQWAQDEMEIGY

SEQ ID NO: 36 - protein, 17 aa, Artificial Sequence
  peptide
EENMDDQWMADEMEIGY

SEQ ID NO: 37 - protein, 17 aa, Artificial Sequence
  peptide
EENMDDQWMQAEMEIGY

SEQ ID NO: 38 - protein, 17 aa, Artificial Sequence
  peptide
EENMDDQWMQDAMEIGY

SEQ ID NO: 39 - protein, 17 aa, Artificial Sequence
  peptide
EENMDDQWMQDEAEIGY

SEQ ID NO: 40 - protein, 17 aa, Artificial Sequence
  peptide
EENMDDQWMQDEMAIGY

SEQ ID NO: 41 - protein, 17 aa, Artificial Sequence
  peptide
EENMDDQWMQDEMEAGY

SEQ ID NO: 42 - protein, 17 aa, Artificial Sequence
  peptide
EENMDDQWMQDEMEIAY

SEQ ID NO: 43 - protein, 17 aa, Artificial Sequence
  peptide
EENMDDQWMQDEMEIGA

SEQ ID NO: 44 - protein, 17 aa, Artificial Sequence
  peptide
AAAMDDQWMQDEMEIGY

SEQ ID NO: 45 - protein, 17 aa, Artificial Sequence
  peptide
EENAAAQWMQDEMEIGY

SEQ ID NO: 46 - protein, 17 aa, Artificial Sequence
  peptide
EENMDDAAAQDEMEIGY

SEQ ID NO: 47 - protein, 17 aa, Artificial Sequence
  peptide
EENMDDQWMAAAMEIGY

SEQ ID NO: 48 - protein, 17 aa, Artificial Sequence
  peptide
EENMDDQWMQDEAAAGY

SEQ ID NO: 49 - protein, 17 aa, Artificial Sequence
  peptide
EENMDDQWMQDEMEIAA

SEQ ID NO: 50 - protein, 5 aa, chicken
SYGMG

SEQ ID NO: 51 - protein, 17 aa, chicken
AIRNDGSWTGYGAAVKG

SEQ ID NO: 52 - protein, 11 aa, chicken
TTGSRGGSIDA

SEQ ID NO: 53 - protein, 9 aa, chicken
SGGGRYYYG

SEQ ID NO: 54 - protein, 7 aa, chicken
ANDKRPS

SEQ ID NO: 55 - protein, 9 aa, chicken
GSAETSSYV

SEQ ID NO: 56 - protein, 5 aa, chicken
SYGMG

SEQ ID NO: 57 - protein, 17 aa, chicken
AIRNDGSWTGYGSAVKG

SEQ ID NO: 58 - protein, 11 aa, chicken
TSGSSGGSVDA

SEQ ID NO: 59 - protein, 9 aa, chicken
SGGGRYYYG

SEQ ID NO: 60 - protein, 7 aa, chicken
ANDKRPS

SEQ ID NO: 61 - protein, 9 aa, chicken
GSAETSSYV

SEQ ID NO: 62 - protein, 5 aa, chicken
SYGME

SEQ ID NO: 63 - protein, 17 aa, chicken
AIRNDGSWTGYGAAVKG

SEQ ID NO: 64 - protein, 11 aa, chicken
TTGSSGGSIDA

SEQ ID NO: 65 - protein, 9 aa, chicken
SGGGNYYYG

SEQ ID NO: 66 - protein, 7 aa, chicken
ANDKRPS

SEQ ID NO: 67 - protein, 9 aa, chicken
GTADTGKYV

SEQ ID NO: 68 - protein, 5 aa, chicken
TYAMG

SEQ ID NO: 69 - protein, 17 aa, chicken
AIRNDGSWTGYGAAVKG

SEQ ID NO: 70 - protein, 11 aa, chicken
YTGSSGGSIGA

SEQ ID NO: 71 - protein, 10 aa, chicken
SGGNRNYYYG

SEQ ID NO: 72 - protein, 7 aa, chicken
ANDKRPS

SEQ ID NO: 73 - protein, 9 aa, chicken
GTADTGKYV

SEQ ID NO: 74 - protein, 5 aa, chicken
TYAMG

SEQ ID NO: 75 - protein, 17 aa, chicken
AIRNDGSWTGYGAAVKG

SEQ ID NO: 76 - protein, 11 aa, chicken
YTGSSGGSIGA

SEQ ID NO: 77 - protein, 9 aa, chicken
SGGGRYYYG

SEQ ID NO: 78 - protein, 7 aa, chicken
ANDKRPS

SEQ ID NO: 79 - protein, 9 aa, chicken
GSAETSSYV

SEQ ID NO: 80 - protein, 5 aa, chicken
TYAMG

SEQ ID NO: 81 - protein, 17 aa, chicken
AIRNDGSWTGYGAAVKG

SEQ ID NO: 82 - protein, 11 aa, chicken
YTGSSGGSIGA

SEQ ID NO: 83 - protein, 10 aa, chicken
SGGSGRYYYG

SEQ ID NO: 84 - protein, 7 aa, chicken
SSTHRPS

SEQ ID NO: 85 - protein, 9 aa, chicken
GTADSSSYV

SEQ ID NO: 86 - protein, 30 aa, chicken
AVTLDESGGGLQTPGGALSLVCKASGFDFS

SEQ ID NO: 87 - protein, 14 aa, chicken
WMRQAPGKGLEYVA

SEQ ID NO: 88 - protein, 32 aa, chicken
HATISRDNGQSTVRLQLNNLRAEDTGTYYCAK

SEQ ID NO: 89 - protein, 10 aa, chicken
WGHGTEVIVS

SEQ ID NO: 90 - protein, 20 aa, chicken
ASTQPSSVSANLGGTVEITC

SEQ ID NO: 91 - protein, 16 aa, chicken
WYQQKSPGSAPVTVIY

SEQ ID NO: 92 - protein, 31 aa, chicken
DIPSRFSGSKSGSTGTLTITGVQAEDEAVYF

SEQ ID NO: 93 - protein, 10 aa, chicken
FGAGTTLTVL

SEQ ID NO: 94 - protein, 30 aa, chicken
AVTLDESGGGLQTPGGTLSLVCKGSGFTFS

SEQ ID NO: 95 - protein, 14 aa, chicken
WMRQAPGKGLEYVA

SEQ ID NO: 96 - protein, 32 aa, chicken
RATISRDNGQSTVRLQLNNLRAEDTATYYCAK

SEQ ID NO: 97 - protein, 10 aa, chicken
WGHGTEVIVS

SEQ ID NO: 98 - protein, 20 aa, chicken
ASTQPSSVSANLGGTVEITC

SEQ ID NO: 99 - protein, 16 aa, chicken
WYQQKSPGSAPVTVIY

SEQ ID NO: 100 - protein, 32 aa, chicken
DIPSRFSGSKSGSTGTLTITGVQAEDEAVYFC

SEQ ID NO: 101 - protein, 10 aa, chicken
FGAGTTLTVL

SEQ ID NO: 102 - protein, 30 aa, chicken
AVTLDESGGGLQTPGGALSLVCKASGFTFS

SEQ ID NO: 103 - protein, 14 aa, chicken
WVRQAPGKGLEYVA

SEQ ID NO: 104 - protein, 32 aa, chicken
RATISRDDGQSTLRLQLNNLRAEDTATYYCAK

SEQ ID NO: 105 - protein, 10 aa, chicken
WGHGTEVIVS

SEQ ID NO: 106 - protein, 20 aa, chicken
ASTQPSSVSANLGETVKITC

SEQ ID NO: 107 - protein, 16 aa, chicken
WYQQKSPGSAPVTLIY

SEQ ID NO: 108 - protein, 32 aa, chicken
NIPSRFSGSKSGSTGTLTITGVQAEDEAVYFC

SEQ ID NO: 109 - protein, 10 aa, chicken
FGAGTTLTVL

SEQ ID NO: 110 - protein, 30 aa, chicken; identical to SEQ ID NO: 102

SEQ ID NO: 111 - protein, 14 aa, chicken
WMRQAPGKGLEYVA

SEQ ID NO: 112 - protein, 32 aa, chicken
RATILRDNGQSTVRLQLSNLRAEDTGTYYCAK

SEQ ID NO: 113 - protein, 10 aa, chicken
WGHGTEVIVS

SEQ ID NO: 114 - protein, 19 aa, chicken
ASTQPSSVSANLGGTVEIT

SEQ ID NO: 115 - protein, 16 aa, chicken
WYQQKSPGSAPVTLIY

SEQ ID NO: 116 - protein, 31 aa, chicken
NIPSRFSGSKSGSTGTLTITGVQAEDEAVYF

SEQ ID NO: 117 - protein, 10 aa, chicken
FGAGTTLTVL

SEQ ID NO: 118 - protein, 30 aa, chicken; identical to SEQ ID NO: 102

SEQ ID NO: 119 - protein, 14 aa, chicken
WMRQAPGKGLEYVA

SEQ ID NO: 120 - protein, 32 aa, chicken; identical to SEQ ID NO: 112

SEQ ID NO: 121 - protein, 10 aa, chicken
WGHGTEVIVS

SEQ ID NO: 122 - protein, 20 aa, chicken
AVTQPASVSANLGGTVEITC

SEQ ID NO: 123 - protein, 16 aa, chicken
WYQQKSPGSAPVTVIY

SEQ ID NO: 124 - protein, 32 aa, chicken; identical to SEQ ID NO: 100

SEQ ID NO: 125 - protein, 10 aa, chicken
FGAGTTLTVL

SEQ ID NO: 126 - protein, 30 aa, chicken; identical to SEQ ID NO: 102

SEQ ID NO: 127 - protein, 14 aa, chicken
WMRQAPGKGLEYVA

SEQ ID NO: 128 - protein, 32 aa, chicken; identical to SEQ ID NO: 112

SEQ ID NO: 129 - protein, 10 aa, chicken
WGHGTEVIVS

SEQ ID NO: 130 - protein, 20 aa, chicken
ASTQPSSVSANPGGTVEITC

SEQ ID NO: 131 - protein, 16 aa, chicken
WYQQKSPGSAPVTVIY

SEQ ID NO: 132 - protein, 32 aa, chicken
NIPSRFSGSKSGSTATLTITGVQAEDEAVYFC

SEQ ID NO: 133 - protein, 10 aa, chicken
FGAGTTLTVL

SEQ ID NO: 134 - protein, 15 aa, Artificial Sequence
  linker
GGGGSGGGGSGGGGS

SEQ ID NO: 135 - DNA, 379 bp, Artificial Sequence
  Variable region
ggcgcgccgaggtgcagctgttggagtctgggggaggcttggtacagcctggggggtccctgagactctcctgtgcagcctctggattcaccttcagcacttatgccatgggttgggtccgccaggcgcccggcaaggggctggagttcgtcgccgctattaggaatgatggtagttggacaggctacggggcggcggtgaagggccgtttcaccatctccagagacaattccaagaacacgctctatctgcaaatgaacagcctgagagcagaggacacggctgtgtattactgcgccaaatatactggtagtagtggtggtagcatcggcgcatggggccagggaaccctggtcaccgtctcctcaggtgaggatcc

SEQ ID NO: 136 - DNA, 379 bp, Artificial Sequence
  Variable region
ggcgcgccgaggtgcagctgttggagtctgggggaggcttggtacagcctggggggtccctgagactctcctgtgcagcctctggattcaccttcagcacttatgccatgggttgggtccgccaggcgcccggcaaggggctggagttcgtcagcgctattaggaatgatggtagttggacaggctacggggcggcggtgaagggccgtttcaccatctccagagacaattccaagaacacggtatatctgcaaatgaacagcctgagagcagaggacacggctgtgtattactgcgccaaatatactggtagtagtggtggtagcatcggcgcatggggccagggaaccctggtcaccgtctcctcaggtgaggatcc

SEQ ID NO: 137 - DNA, 379 bp, Artificial Sequence
  Variable region
ggcgcgccgaggtgcagctgttggagtctgggggaggcttggtacagcctggggggtccctgagactctcctgtgcagcctctggattcaccttcagcacttatgccatgggttgggtccgccaggcgcccggcaaggggctggagttcgtcgctgctattaggaatgatggtagttggacaggctacggggcggcggtgaagggccgtgtcaccatctccagagacaattccaagaacacggtatatctgcaaatgaacagcctgagagcagaggacacggctgtgtattactgcgccaaatatactggtagtagtggtggtagcatcggcgcatggggccagggaaccctggtcaccgtctcctcaggtgaggatcc

SEQ ID NO: 138 - DNA, 336 bp, Artificial Sequence
  Variable region
ggcgcgccagctatgagctgactcagccaccctcggtgtcagtgtccccaggacagacggccaggatcacctgctccggggggaataggaactactactatggctggtaccagcagaagccaggccaggcccctgtgctggtgatatatgctaacgacaagagaccctcgggaatccctgagcgattctctggctcctcatcagggacaacagtgacgttgaccatcagtggagtccaggcagaagatgaggctgactattactgtgggaccgcagacaccgggaagtatgtattcggcggagggaccaagctgaccgtcctgggtgagtggatcc

SEQ ID NO: 139 - DNA, 336 bp, Artificial Sequence
  Variable region
ggcgcgccagctatgagctgactcagccaccctcggtgtcagtgtccccaggacagacggccaggatcacctgctccggggggaataggaactactactatggctggtaccagcagaagccaggccaggcccctgtgaccgtgatatatgctaacgacaagagaccctcgggaatccctgagcgattctctggctcctactcagggaacacaaccacgttgaccatcagtggagtccaggcagaagatgaggctgactattactgtgggaccgcagacaccgggaagtatgtattcggcggagggaccaagctgaccgtcctgggtgagtggatcc

SEQ ID NO: 140 - DNA, 336 bp, Artificial Sequence
  Variable region
ggcgcgccagctatgagctgactcagccaccctcggtgtcagtgtccccaggacagacggccaggatcacctgctccggggggaataggaactactactatggctggtaccagcagaagccaggccaggcccctgtgaccgtgatatatgctaacgacaagagaccctcgggaatccctgagcgattctctggctccacctcagggaacacaaccacgttgaccatcagtggagtccaggcagaagatgaggctgactattactgtgggaccgcagacaccgggaagtatgtattcggcggagggaccaagctgaccgtcctgggtgagtggatcc

SEQ ID NO: 141 - DNA, 336 bp, Artificial Sequence
  Variable region
ggcgcgccagctatgagctgactcagccaccctcggtgtcagtgtccccaggacagacggccaggatcacctgctccggggggaataggaactactactatggctggtaccagcagaagccaggccaggcccctgtgaccgtgatatatgctaacgacaagagaccctcgggaatccctgagcgattctctggctccaactcagggtcaacaaccacgttgaccatcagtggagtccaggcagaagatgaggctgactattactgtgggaccgcagacaccgggaagtatgtattcggcggagggaccaagctgaccgtcctgggtgagtggatcc

SEQ ID NO: 142 - DNA, 336 bp, Artificial Sequence
  Variable region
ggcgcgccagctatgagctgactcagccaccctcggtgtcagtgtccccaggacagacggccaggatcacctgctccgggggtagtggcaggtactattatggctggtaccagcagaagccaggccaggcccctgtgctggtgatatatagcagcacccacagaccctcaggaatccctgagcgattctctggctcctcatcagggacaacagtgacgttgaccatcagtggagtccaggcagaagatgaggctgactattactgtgggactgcagacagcagcagctatgtcttcggcggagggaccaagctgaccgtcctgggtgagtggatcc

SEQ ID NO: 143 - DNA, 336 bp, Artificial Sequence
  Variable region
ggcgcgccagctatgagctgactcagccaccctcggtgtcagtgtccccaggacagacggccaggatcacctgctccgggggtagtggcaggtactattatggctggtaccagcagaagccaggccaggcccctgtgaccgtgatatatagcagcacccacagaccctcaggaatccctgagcgattctctggctcctattcagggaatacaaccacgttgaccatcagtggagtccaggcagaagatgaggctgactattactgtgggactgcagacagcagcagctatgtcttcggcggagggaccaagctgaccgtcctgggtgagtggatcc

SEQ ID NO: 144 - DNA, 336 bp, Artificial Sequence
  Variable region
ggcgcgccagctatgagctgactcagccaccctcggtgtcagtgtccccaggacagacggccaggatcacctgctccgggggtagtggcaggtactattatggctggtaccagcagaagccaggccaggcccctgtgaccgtgatatatagcagcacccacagaccctcaggaatccctgagcgattctctggctccaattcagggaatacaaccacgttgaccatcagtggagtccaggcagaagatgaggctgactattactgtgggactgcagacagcagcagctatgtcttcggcggagggaccaagctgaccgtcctgggtgagtggatcc

SEQ ID NO: 145 - DNA, 336 bp, Artificial Sequence
  Variable region
ggcgcgccagctatgagctgactcagccaccctcggtgtcagtgtccccaggacagacggccaggatcacctgctccgggggtagtggcaggtactattatggctggtaccagcagaagccaggccaggcccctgtgaccgtgatatatagcagcacccacagaccctcaggaatccctgagcgattctctggctccacctcagggaatacaaccacgttgaccatcagtggagtccaggcagaagatgaggctgactattactgtgggactgcagacagcagcagctatgtcttcggcggagggaccaagctgaccgtcctgggtgagtggatcc

SEQ ID NO: 146 - DNA, 336 bp, Artificial Sequence
  Variable region
ggcgcgccagctatgagctgactcagccaccctcggtgtcagtgtccccaggacagacggccaggatcacctgctccgggggtagtggcaggtactattatggctggtaccagcagaagccaggccaggcccctgtgaccgtgatatatagcagcacccacagaccctcaggaatccctgagcgattctctggctccaattcagggagcacaaccacgttgaccatcagtggagtccaggcagaagatgaggctgactattactgtgggactgcagacagcagcagctatgtcttcggcggagggaccaagctgaccgtcctgggtgagtggatcc

SEQ ID NO: 147 - DNA, 31 bp, Artificial Sequence
  Primer
atataggcgcgccgaggtgcagctgttggag

SEQ ID NO: 148 - DNA, 30 bp, Artificial Sequence
  Primer
tatatggatcctcacctgaggagacggtga

SEQ ID NO: 149 - DNA, 34 bp, Artificial Sequence
  Primer
atataggcgcgccagctatgagctgactcagcca

SEQ ID NO: 150 - DNA, 30 bp, Artificial Sequence
  Primer
tatatggatccactcacccaggacggtcag

SEQ ID NO: 151 - DNA, 379 bp, Artificial Sequence
  Variable region
ggcgcgccgaggtgcagctgttggagtctgggggaggcttggtacagcctggggggtccctgagactctcctgtgcagcctctggattcaccttcagcagttatggcatgggatgggtccgccaggcgcccggcaaggggctggagttcgtcgccgctattaggaatgatggcagttggacaggctacggggcggcggtgaagggccgtttcaccatctccagagacaattccaagaacacgctctatctgcaaatgaacagcctgagagcagaggacacggctgtgtattactgcgccaaaactactggtagtcgtggtggtagcatcgacgcatggggccagggaaccctggtcaccgtctcctcaggtgaggatcc

SEQ ID NO: 152 - DNA, 333 bp, Artificial Sequence
  Variable region
ggcgcgccagctatgagctgactcagccaccctcggtgtcagtgtccccaggacagacggccaggatcacctgctccgggggtggcaggtactattatggctggtaccagcagaagccaggccaggcccctgtgaccgtgatatatgctaacgacaagagaccctcgggaatccctgagcgattctctggctccaactcagggtcaacaaccacgttgaccatcagtggagtccaggcagaagatgaggctgactattactgtgggagtgcagagaccagcagctatgtattcggcggagggaccaagctgaccgtcctgggtgagtggatcc

SEQ ID NO: 153 - protein, 330 aa, Artificial Sequence [sequence omitted]

SEQ ID NO: 154 - protein, 107 aa, Artificial Sequence
  Light chain constant region
GTVAAPSVFIFPPSDEQLKSGTASVVCLLNNFYPREAKVQWKVDNALQSGNSQESVTEQDSKDSTYSLSSTLTLSKADYEKHKVYACEVTHQGLSSPVTKSFNRGEC

SEQ ID NO: 155 - protein, 120 aa, Artificial Sequence
  Variable region
EVQLLESGGGLVQPGGSLRLSCAASGFTFSTYAMGWVRQAPGKGLEFVAAIRNDGSWTGYGAAVKGRFTISRDNSKNTLYLQMNSLRAEDTAVYYCAKYTGSSGGSIGAWGQGTLVTVSS

SEQ ID NO: 156 - protein, 120 aa, Artificial Sequence
  Variable region
EVQLLESGGGLVQPGGSLRLSCAASGFTFSTYAMGWVRQAPGKGLEFVSAIRNDGSWTGYGAAVKGRFTISRDNSKNTVYLQMNSLRAEDTAVYYCAKYTGSSGGSIGAWGQGTLVTVSS

SEQ ID NO: 157 - protein, 120 aa, Artificial Sequence
  Variable region
EVQLLESGGGLVQPGGSLRLSCAASGFTFSTYAMGWVRQAPGKGLEFVAAIRNDGSWTGYGAAVKGRVTISRDNSKNTVYLQMNSLRAEDTAVYYCAKYTGSSGGSIGAWGQGTLVTVSS

SEQ ID NO: 158 - protein, 105 aa, Artificial Sequence
  Variable region
SYELTQPPSVSVSPGQTARITCSGGNRNYYYGWYQQKPGQAPVLVIYANDKRPSGIPERFSGSSSGTTVTLTISGVQAEDEADYYCGTADTGKYVFGGGTKLTVL

SEQ ID NO: 159 - protein, 105 aa, Artificial Sequence
  Variable region
SYELTQPPSVSVSPGQTARITCSGGNRNYYYGWYQQKPGQAPVTVIYANDKRPSGIPERFSGSYSGNTTTLTISGVQAEDEADYYCGTADTGKYVFGGGTKLTVL

SEQ ID NO: 160 - protein, 105 aa, Artificial Sequence
  Variable region
SYELTQPPSVSVSPGQTARITCSGGNRNYYYGWYQQKPGQAPVTVIYANDKRPSGIPERFSGSTSGNTTTLTISGVQAEDEADYYCGTADTGKYVFGGGTKLTVL

SEQ ID NO: 161 - protein, 105 aa, Artificial Sequence
  Variable region
SYELTQPPSVSVSPGQTARITCSGGNRNYYYGWYQQKPGQAPVTVIYANDKRPSGIPERFSGSNSGSTTTLTISGVQAEDEADYYCGTADTGKYVFGGGTKLTVL

SEQ ID NO: 162 - protein, 120 aa, Artificial Sequence; identical to SEQ ID NO: 155
  Variable region

SEQ ID NO: 163 - protein, 120 aa, Artificial Sequence; identical to SEQ ID NO: 156
  Variable region

SEQ ID NO: 164 - protein, 120 aa, Artificial Sequence; identical to SEQ ID NO: 157
  Variable region

SEQ ID NO: 165 - protein, 105 aa, Artificial Sequence
  Variable region
SYELTQPPSVSVSPGQTARITCSGGSGRYYYGWYQQKPGQAPVLVIYSSTHRPSGIPERFSGSSSGTTVTLTISGVQAEDEADYYCGTADSSSYVFGGGTKLTVL

SEQ ID NO: 166 - protein, 105 aa, Artificial Sequence
  Variable region
SYELTQPPSVSVSPGQTARITCSGGSGRYYYGWYQQKPGQAPVTVIYSSTHRPSGIPERFSGSYSGNTTTLTISGVQAEDEADYYCGTADSSSYVFGGGTKLTVL

SEQ ID NO: 167 - protein, 105 aa, Artificial Sequence
  Variable region
SYELTQPPSVSVSPGQTARITCSGGSGRYYYGWYQQKPGQAPVTVIYSSTHRPSGIPERFSGSNSGNTTTLTISGVQAEDEADYYCGTADSSSYVFGGGTKLTVL

SEQ ID NO: 168 - protein, 105 aa, Artificial Sequence
  Variable region
SYELTQPPSVSVSPGQTARITCSGGSGRYYYGWYQQKPGQAPVTVIYSSTHRPSGIPERFSGSTSGNTTTLTISGVQAEDEADYYCGTADSSSYVFGGGTKLTVL

SEQ ID NO: 169 - protein, 105 aa, Artificial Sequence
  Variable region
SYELTQPPSVSVSPGQTARITCSGGSGRYYYGWYQQKPGQAPVTVIYSSTHRPSGIPERFSGSNSGSTTTLTISGVQAEDEADYYCGTADSSSYVFGGGTKLTVL

SEQ ID NO: 170 - protein, 450 aa, Artificial Sequence
  Heavy chain
EVQLLESGGGLVQPGGSLRLSCAASGFTFSSYGMGWVRQAPGKGLEFVAAIRNDGSWTGYGAAVKGRFTISRDNSKNTLYLQMNSLRAEDTAVYYCAKTTGSRGGSIDAWGQGTLVTVSSASTKGPSVFPLAPSSKSTSGGTAALGCLVKDYFPEPVTVSWNSGALTSGVHTFPAVLQSSGLYSLSSVVTVPSSSLGTQTYICNVNHKPSNTKVDKKVEPKSCDKTHTCPPCPAPELLGGPSVFLFPPKPKDTLMISRTPEVTCVVVDVSHEDPEVKFNWYVDGVEVHNAKTKPREEQYNSTYRVVSVLTVLHQDWLNGKEYKCKVSNKALPAPIEKTISKAKGQPREPQVYTLPPSRDELTKNQVSLTCLVKGFYPSDIAVEWESNGQPENNYKTTPPVLDSDGSFFLYSKLTVDKSRWQQGNVFSCSVMHEALHNHYTQKSLSLSPGK

SEQ ID NO: 171 - protein, 211 aa, Artificial Sequence
  Light chain
SYELTQPPSVSVSPGQTARITCSGGGRYYYGWYQQKPGQAPVTVIYANDKRPSGIPERFSGSNSGSTTTLTISGVQAEDEADYYCGSAETSSYVFGGGTKLTVLGTVAAPSVFIFPPSDEQLKSGTASVVCLLNNFYPREAKVQWKVDNALQSGNSQESVTEQDSKDSTYSLSSTLTLSKADYEKHKVYACEVTHQGLSSPVTKSFNRGEC

SEQ ID NO: 172 - protein, 450 aa, Artificial Sequence
  Heavy chain
EVQLLESGGGLVQPGGSLRLSCAASGFTFSTYAMGWVRQAPGKGLEFVAAIRNDGSWTGYGAAVKGRFTISRDNSKNTLYLQMNSLRAEDTAVYYCAKYTGSSGGSIGAWGQGTLVTVSSASTKGPSVFPLAPSSKSTSGGTAALGCLVKDYFPEPVTVSWNSGALTSGVHTFPAVLQSSGLYSLSSVVTVPSSSLGTQTYICNVNHKPSNTKVDKKVEPKSCDKTHTCPPCPAPELLGGPSVFLFPPKPKDTLMISRTPEVTCVVVDVSHEDPEVKFNWYVDGVEVHNAKTKPREEQYNSTYRVVSVLTVLHQDWLNGKEYKCKVSNKALPAPIEKTISKAKGQPREPQVYTLPPSRDELTKNQVSLTCLVKGFYPSDIAVEWESNGQPENNYKTTPPVLDSDGSFFLYSKLTVDKSRWQQGNVFSCSVMHEALHNHYTQKSLSLSPGK

SEQ ID NO: 173 - protein, 212 aa, Artificial Sequence
  Light chain
SYELTQPPSVSVSPGQTARITCSGGNRNYYYGWYQQKPGQAPVTVIYANDKRPSGIPERFSGSNSGSTTTLTISGVQAEDEADYYCGTADTGKYVFGGGTKLTVLGTVAAPSVFIFPPSDEQLKSGTASVVCLLNNFYPREAKVQWKVDNALQSGNSQESVTEQDSKDSTYSLSSTLTLSKADYEKHKVYACEVTHQGLSSPVTKSFNRGEC

SEQ ID NO: 174 - protein, 450 aa, Artificial Sequence; identical to SEQ ID NO: 172
  Heavy chain

SEQ ID NO: 175 - protein, 211 aa, Artificial Sequence; identical to SEQ ID NO: 171
  Light chain

SEQ ID NO: 176 - protein, 450 aa, Artificial Sequence; identical to SEQ ID NO: 172
  Heavy chain

SEQ ID NO: 177 - protein, 212 aa, Artificial Sequence
  Light chain
SYELTQPPSVSVSPGQTARITCSGGSGRYYYGWYQQKPGQAPVTVIYSSTHRPSGIPERFSGSNSGSTTTLTISGVQAEDEADYYCGTADSSSYVFGGGTKLTVLGTVAAPSVFIFPPSDEQLKSGTASVVCLLNNFYPREAKVQWKVDNALQSGNSQESVTEQDSKDSTYSLSSTLTLSKADYEKHKVYACEVTHQGLSSPVTKSFNRGEC

SEQ ID NO: 178 - DNA, 360 bp, Artificial Sequence
  Variable region
gaggtgcagctgttggagtctgggggaggactggtgcagcctggcggaagcctgagactgtcttgtgccgccagcggcttcaccttcagcacctatgccatgggctgggtgcgccaggcccctggaaagggcctggaatttgtggccgccatccggaacgatggcagctggacaggatatggcgccgctgtgaagggccggttcaccatcagccgggacaacagcaagaacaccctgtacctgcagatgaacagcctgcgggccgaggacaccgccgtgtactactgtgccaagtacaccggcagcagcggcggctctattggagcttggggacagggaaccctggtcaccgtctcctca

SEQ ID NO: 179 - DNA, 984 bp, Artificial Sequence
  Heavy chain constant region
gccagcaccaagggccccagcgtgttccctctggccccttgtagcagaagcaccagcgagtctacagccgccctgggctgcctcgtgaaggactactttcccgagcccgtgaccgtgtcctggaactctggcgctctgacaagcggcgtgcacacctttccagccgtgctgcagagcagcggcctgtactctctgagcagcgtcgtgactgtgcccagcagctctctgggcaccaagacctacacctgtaacgtggaccacaagcccagcaacaccaaggtggacaagcgggtggaatctaagtacggccctccctgccctccttgcccagcccctgaatttctgggcggaccctccgtgttcctgttccccccaaagcccaaggacaccctgatgatcagccggacccccgaagtgacctgcgtggtggtggatgtgtcccaggaagatcccgaggtgcagttcaattggtacgtggacggcgtggaagtgcacaacgccaagaccaagcctagagaggaacagttcaacagcacctaccgggtggtgtccgtgctgacagtgctgcatcaggactggctgaacggcaaagagtacaagtgcaaggtgtccaacaagggcctgcccagctccatcgagaaaaccatcagcaaggccaagggccagccccgcgaaccccaggtgtacacactgcctccaagccaggaagagatgaccaagaaccaggtgtccctgacctgtctcgtgaaaggcttctacccctccgatatcgccgtggaatgggagagcaacggccagcccgagaacaactacaagacaaccccccctgtgctggacagcgacggctcattcttcctgtacagcagactgaccgtggacaagagccggtggcaggaaggcaacgtgttcagctgcagcgtgatgcacgaggccctgcacaaccactacacccagaagtccctgtctctgagcctgggcaagtga

SEQ ID NO: 180 - DNA, 315 bp, Artificial Sequence
  Variable region
agctatgagctgactcagccaccctcggtgtcagtgtctcctggccagaccgccagaatcacatgtagcggcggcagcggccggtactactacggctggtatcagcagaagcccggccaggcccctgtgaccgtgatctacagcagcacccacagacccagcggcatccccgagagattcagcggcagcaatagcggctccaccaccaccctgacaatcagcggagtgcaggccgaggacgaggccgattactactgtggcaccgccgacagcagcagctacgtgttcggcggaggaaccaagctgaccgtcctg

SEQ ID NO: 181 - protein, 321 aa, Artificial Sequence
  Light chain constant region
GGTCAGCCCAAGGCTGCCCCCTCGGTCACTCTGTTCCCGCCCTCCTCTGAGGAGCTTCAAGCCAACAAGGCCACACTGGTGTGTCTCATAAGTGACTTCTACCCGGGAGCCGTGACAGTGGCCTGGAAGGCAGATAGCAGCCCCGTCAAGGCGGGAGTGGAGACCACCACACCCTCCAAACAAAGCAACAACAAGTACGCGGCCAGCAGCTATCTGAGCCTGACGCCTGAGCAGTGGAAGTCCCACAGAAGCTACAGCTGCCAGGTCACGCATGAAGGGAGCACCGTGGAGAAGACAGTGGCCCCTACAGAATGTTCATAG

SEQ ID NO: 182 - protein, 120 aa, Artificial Sequence; identical to SEQ ID NO: 155
  Variable region

SEQ ID NO: 183 - protein, 327 aa, Artificial Sequence
  Heavy chain constant region
ASTKGPSVFPLAPCSRSTSESTAALGCLVKDYFPEPVTVSWNSGALTSGVHTFPAVLQSSGLYSLSSVVTVPSSSLGTKTYTCNVDHKPSNTKVDKRVESKYGPPCPPCPAPEFLGGPSVFLFPPKPKDTLMISRTPEVTCVVVDVSQEDPEVQFNWYVDGVEVHNAKTKPREEQFNSTYRVVSVLTVLHQDWLNGKEYKCKVSNKGLPSSIEKTISKAKGQPREPQVYTLPPSQEEMTKNQVSLTCLVKGFYPSDIAVEWESNGQPENNYKTTPPVLDSDGSFFLYSRLTVDKSRWQEGNVFSCSVMHEALHNHYTQKSLSLSLGK

SEQ ID NO: 184 - protein, 105 aa, Artificial Sequence; identical to SEQ ID NO: 169
  Variable region

SEQ ID NO: 185 - protein, 106 aa, Artificial Sequence
  Light chain constant region
GQPKAAPSVTLFPPSSEELQANKATLVCLISDFYPGAVTVAWKADSSPVKAGVETTTPSKQSNNKYAASSYLSLTPEQWKSHRSYSCQVTHEGSTVEKTVAPTECS

SEQ ID NO: 186 - protein, 120 aa, Artificial Sequence
  Variable region
EVQLLESGGGLVQPGGSLRLSCAASGFTFSSYGMGWVRQAPGKGLEFVAAIRNDGSWTGYGAAVKGRFTISRDNSKNTLYLQMNSLRAEDTAVYYCAKTTGSRGGSIDAWGQGTLVTVSS

SEQ ID NO: 187 - protein, 104 aa, Artificial Sequence
  Variable region
SYELTQPPSVSVSPGQTARITCSGGGRYYYGWYQQKPGQAPVTVIYANDKRPSGIPERFSGSNSGSTTTLTISGVQAEDEADYYCGSAETSSYVFGGGTKLTVL

SEQ ID NO: 188 - protein, 120 aa, Artificial Sequence; identical to SEQ ID NO: 155
  Variable region

SEQ ID NO: 189 - protein, 105 aa, Artificial Sequence; identical to SEQ ID NO: 161
  Variable region

SEQ ID NO: 190 - protein, 120 aa, Artificial Sequence; identical to SEQ ID NO: 155
  Variable region

SEQ ID NO: 191 - protein, 104 aa, Artificial Sequence; identical to SEQ ID NO: 187
  Variable region

SEQ ID NO: 192 - protein, 120 aa, Artificial Sequence; identical to SEQ ID NO: 155
  Variable region

SEQ ID NO: 193 - protein, 105 aa, Artificial Sequence; identical to SEQ ID NO: 169
  Variable region

SEQ ID NO: 194 - protein, 120 aa, Artificial Sequence; identical to SEQ ID NO: 155
  Variable region

SEQ ID NO: 195 - protein, 105 aa, Artificial Sequence; identical to SEQ ID NO: 169
  Variable region

SEQ ID NO: 196 - protein, 447 aa, Artificial Sequence
  Heavy chain
EVQLLESGGGLVQPGGSLRLSCAASGFTFSTYAMGWVRQAPGKGLEFVAAIRNDGSWTGYGAAVKGRFTISRDNSKNTLYLQMNSLRAEDTAVYYCAKYTGSSGGSIGAWGQGTLVTVSSASTKGPSVFPLAPCSRSTSESTAALGCLVKDYFPEPVTVSWNSGALTSGVHTFPAVLQSSGLYSLSSVVTVPSSSLGTKTYTCNVDHKPSNTKVDKRVESKYGPPCPPCPAPEFLGGPSVFLFPPKPKDTLMISRTPEVTCVVVDVSQEDPEVQFNWYVDGVEVHNAKTKPREEQFNSTYRVVSVLTVLHQDWLNGKEYKCKVSNKGLPSSIEKTISKAKGQPREPQVYTLPPSQEEMTKNQVSLTCLVKGFYPSDIAVEWESNGQPENNYKTTPPVLDSDGSFFLYSRLTVDKSRWQEGNVFSCSVMHEALHNHYTQKSLSLSLGK

SEQ ID NO: 197 - protein, 211 aa, Artificial Sequence
  Light chain
SYELTQPPSVSVSPGQTARITCSGGSGRYYYGWYQQKPGQAPVTVIYSSTHRPSGIPERFSGSNSGSTTTLTISGVQAEDEADYYCGTADSSSYVFGGGTKLTVLGQPKAAPSVTLFPPSSEELQANKATLVCLISDFYPGAVTVAWKADSSPVKAGVETTTPSKQSNNKYAASSYLSLTPEQWKSHRSYSCQVTHEGSTVEKTVAPTECS